European Patent Specification EP 4 196 488 B1, published August 6, 2025. Title: CLEAVABLE LINKER COMPOSITION AND METHODS. Applicant: JANUX THERAPEUTICS, INC. The sequence listing filed with the application follows.

SEQUENCE LISTING (27 sequences)

SEQ ID NO: 1 - protein, 8 aa, Artificial Sequence
  Description of Artificial Sequence: Synthetic peptide
LSGRSDAG

SEQ ID NO: 2 - protein, 13 aa, Artificial Sequence
  Description of Artificial Sequence: Synthetic peptide
ISSGLLSGRSDNH

SEQ ID NO: 3 - protein, 13 aa, Artificial Sequence
  Description of Artificial Sequence: Synthetic peptide
ISSGLLSGRSDAG

SEQ ID NO: 4 - protein, 18 aa, Artificial Sequence
  Description of Artificial Sequence: Synthetic peptide
AAGLLAPPGGLSGRSDAG

SEQ ID NO: 5 - protein, 12 aa, Artificial Sequence
  Description of Artificial Sequence: Synthetic peptide
SPLGLSGRSDAG

SEQ ID NO: 6 - protein, 15 aa, Artificial Sequence
  Description of Artificial Sequence: Synthetic peptide
LSGRSDAGSPLGLAG

SEQ ID NO: 7 - protein, 21 aa, Artificial Sequence
  Description of Artificial Sequence: Synthetic peptide
QGQSGQLSCEGWAMNREQCRA

SEQ ID NO: 8 - protein, 16 aa, Artificial Sequence
  Description of Artificial Sequence: Synthetic peptide
GGPCRSHIDVAKPICV

SEQ ID NO: 9 - protein, 21 aa, Artificial Sequence
  Description of Artificial Sequence: Synthetic peptide
QGQSGQGYLWGCEWNCGGITT

SEQ ID NO: 10 - protein, 21 aa, Artificial Sequence
  Description of Artificial Sequence: Synthetic peptide
QGQSGSGYLWGCEWNCAGITT

SEQ ID NO: 11 - protein, 115 aa, Artificial Sequence
  Description of Artificial Sequence: Synthetic polypeptide
EVQLVESGGGLVQPGNSLRLSCAASGFTFSKFGMSWVRQAPGKGLEWVSSISGSGRDTLYADSVKGRFTISRDNAKTTLYLQMNSLRPEDTAVYYCTIGGSLSVSSQGTLVTVSS

SEQ ID NO: 12 - protein, 266 aa, Artificial Sequence
  Description of Artificial Sequence: Synthetic polypeptide
QGQSGQLSCEGWAMNREQCRAGSSGGSGGSGGSGISSGLLSGRSDNHGSSGTDILLTQSPVILSVSPGERVSFSCRASQSIGTNIHWYQQRTNGSPRLLIKYASESISGIPSRFSGSGSGTDFTLSINSVESEDIADYYCQQNNNWPTTFGAGTKLELKRTVAAPSVFIFPPSDEQLKSGTASVVCLLNNFYPREAKVQWKVDNALQSGNSQESVTEQDSKDSTYSLSSTLTLSKADYEKHKVYACEVTHQGLSSPVTKSFNRGEC

SEQ ID NO: 13 - protein, 676 aa, Artificial Sequence
  Description of Artificial Sequence: Synthetic polypeptide
EVQLVESGGGLVQPGNSLRLSCAASGFTFSKFGMSWVRQAPGKGLEWVSSISGSGRDTLYADSVKGRFTISRDNAKTTLYLQMNSLRPEDTAVYYCTIGGSLSVSSQGTLVTVSSGGGGSGGGSQGQSGQGYLWGCEWNCGGITTGSSGGSGGSGGISSGLLSGRSDNHGGGSQTVVTQEPSLTVSPGGTVTLTCRSSTGAVTTSNYANWVQQKPGQAPRGLIGGTNKRAPGTPARFSGSLLGGKAALTLSGVQPEDEAEYYCALWYSNLWVFGGGTKLTVLGGGGSGGGGSGGGGSEVQLVESGGGLVQPGGSLKLSCAASGFTFNTYAMNWVRQAPGKGLEWVARIRSKYNNYATYYADSVKDRFTISRDDSKNTAYLQMNNLKTEDTAVYYCVRHGNFGNSYVSWFAYWGQGTLVTVSSGGGGSQVQLKQSGPGLVQPSQSLSITCTVSGFSLTNYGVHWVRQSPGKGLEWLGVIWSGGNTDYNTPFTSRLSINKDNSKSQVFFKMNSLQSNDTAIYYCARALTYYDYEFAYWGQGTLVTVSAASTKGPSVFPLAPSSKSTSGGTAALGCLVKDYFPEPVTVSWNSGALTSGVHTFPAVLQSSGLYSLSSVVTVPSSSLGTQTYICNVNHKPSNTKVDKKVEPKSCGGHHHHHHHHGGGLNDIFEAQKIEWHE

SEQ ID NO: 14 - protein, 255 aa, Artificial Sequence
  Description of Artificial Sequence: Synthetic polypeptide
GGPCRSHIDVAKPICVGGGGSGGSISSGLLSGRSDAGGGGSDILLTQSPVILSVSPGERVSFSCRASQSIGTNIHWYQQRTNGSPRLLIKYASESISGIPSRFSGSGSGTDFTLSINSVESEDIADYYCQQNNNWPTTFGAGTKLELKRTVAAPSVFIFPPSDEQLKSGTASVVCLLNNFYPREAKVQWKVDNALQSGNSQESVTEQDSKDSTYSLSSTLTLSKADYEKHKVYACEVTHQGLSSPVTKSFNRGEC

SEQ ID NO: 15 - protein, 660 aa, Artificial Sequence
  Description of Artificial Sequence: Synthetic polypeptide
EVQLVESGGGLVQPGNSLRLSCAASGFTFSKFGMSWVRQAPGKGLEWVSSISGSGRDTLYADSVKGRFTISRDNAKTTLYLQMNSLRPEDTAVYYCTIGGSLSVSSQGTLVTVSSGGGGSGGGSQGQSGQGYLWGCEWNCAGITTGSSGGSGGSGGISSGLLSGRSDAGGGGSQTVVTQEPSLTVSPGGTVTLTCRSSTGAVTTSNYANWVQQKPGQAPRGLIGGTNKRAPGTPARFSGSLLGGKAALTLSGVQPEDEAEYYCALWYSNLWVFGGGTKLTVLGGGGSGGGGSGGGGSEVQLVESGGGLVQPGGSLKLSCAASGFTFNTYAMNWVRQAPGKGLEWVARIRSKYNNYATYYADSVKDRFTISRDDSKNTAYLQMNNLKTEDTAVYYCVRHGNFGNSYVSWFAYWGQGTLVTVSSGGGGSQVQLKQSGPGLVQPSQSLSITCTVSGFSLTNYGVHWVRQSPGKGLEWLGVIWSGGNTDYNTPFTSRLSINKDNSKSQVFFKMNSLQSNDTAIYYCARALTYYDYEFAYWGQGTLVTVSAASTKGPSVFPLAPSSKSTSGGTAALGCLVKDYFPEPVTVSWNSGALTSGVHTFPAVLQSSGLYSLSSVVTVPSSSLGTQTYICNVNHKPSNTKVDKKVEPKSCAAAHHHHHHHH

SEQ ID NO: 16 - protein, 261 aa, Artificial Sequence
  Description of Artificial Sequence: Synthetic polypeptide
GGPCRSHIDVAKPICVGGGGSSGGSAAGLLAPPGGLSGRSDAGGGGSDILLTQSPVILSVSPGERVSFSCRASQSIGTNIHWYQQRTNGSPRLLIKYASESISGIPSRFSGSGSGTDFTLSINSVESEDIADYYCQQNNNWPTTFGAGTKLELKRTVAAPSVFIFPPSDEQLKSGTASVVCLLNNFYPREAKVQWKVDNALQSGNSQESVTEQDSKDSTYSLSSTLTLSKADYEKHKVYACEVTHQGLSSPVTKSFNRGEC

SEQ ID NO: 17 - protein, 660 aa, Artificial Sequence
  Description of Artificial Sequence: Synthetic polypeptide
EVQLVESGGGLVQPGNSLRLSCAASGFTFSKFGMSWVRQAPGKGLEWVSSISGSGRDTLYADSVKGRFTISRDNAKTTLYLQMNSLRPEDTAVYYCTIGGSLSVSSQGTLVTVSSGGGGSGGGSQGQSGQGYLWGCEWNCAGITTGSSGGSAAGLLAPPGGLSGRSDAGGGGSQTVVTQEPSLTVSPGGTVTLTCRSSTGAVTTSNYANWVQQKPGQAPRGLIGGTNKRAPGTPARFSGSLLGGKAALTLSGVQPEDEAEYYCALWYSNLWVFGGGTKLTVLGGGGSGGGGSGGGGSEVQLVESGGGLVQPGGSLKLSCAASGFTFNTYAMNWVRQAPGKGLEWVARIRSKYNNYATYYADSVKDRFTISRDDSKNTAYLQMNNLKTEDTAVYYCVRHGNFGNSYVSWFAYWGQGTLVTVSSGGGGSQVQLKQSGPGLVQPSQSLSITCTVSGFSLTNYGVHWVRQSPGKGLEWLGVIWSGGNTDYNTPFTSRLSINKDNSKSQVFFKMNSLQSNDTAIYYCARALTYYDYEFAYWGQGTLVTVSAASTKGPSVFPLAPSSKSTSGGTAALGCLVKDYFPEPVTVSWNSGALTSGVHTFPAVLQSSGLYSLSSVVTVPSSSLGTQTYICNVNHKPSNTKVDKKVEPKSCAAAHHHHHHHH

SEQ ID NO: 18 - protein, 255 aa, Artificial Sequence
  Description of Artificial Sequence: Synthetic polypeptide
GGPCRSHIDVAKPICVGGGGSGGGGSPLGLSGRSDAGGGGSDILLTQSPVILSVSPGERVSFSCRASQSIGTNIHWYQQRTNGSPRLLIKYASESISGIPSRFSGSGSGTDFTLSINSVESEDIADYYCQQNNNWPTTFGAGTKLELKRTVAAPSVFIFPPSDEQLKSGTASVVCLLNNFYPREAKVQWKVDNALQSGNSQESVTEQDSKDSTYSLSSTLTLSKADYEKHKVYACEVTHQGLSSPVTKSFNRGEC

SEQ ID NO: 19 - protein, 660 aa, Artificial Sequence
  Description of Artificial Sequence: Synthetic polypeptide
EVQLVESGGGLVQPGNSLRLSCAASGFTFSKFGMSWVRQAPGKGLEWVSSISGSGRDTLYADSVKGRFTISRDNAKTTLYLQMNSLRPEDTAVYYCTIGGSLSVSSQGTLVTVSSGGGGSGGGSQGQSGQGYLWGCEWNCAGITTGSSGGSGGGSGGSPLGLSGRSDAGGGGSQTVVTQEPSLTVSPGGTVTLTCRSSTGAVTTSNYANWVQQKPGQAPRGLIGGTNKRAPGTPARFSGSLLGGKAALTLSGVQPEDEAEYYCALWYSNLWVFGGGTKLTVLGGGGSGGGGSGGGGSEVQLVESGGGLVQPGGSLKLSCAASGFTFNTYAMNWVRQAPGKGLEWVARIRSKYNNYATYYADSVKDRFTISRDDSKNTAYLQMNNLKTEDTAVYYCVRHGNFGNSYVSWFAYWGQGTLVTVSSGGGGSQVQLKQSGPGLVQPSQSLSITCTVSGFSLTNYGVHWVRQSPGKGLEWLGVIWSGGNTDYNTPFTSRLSINKDNSKSQVFFKMNSLQSNDTAIYYCARALTYYDYEFAYWGQGTLVTVSAASTKGPSVFPLAPSSKSTSGGTAALGCLVKDYFPEPVTVSWNSGALTSGVHTFPAVLQSSGLYSLSSVVTVPSSSLGTQTYICNVNHKPSNTKVDKKVEPKSCAAAHHHHHHHH

SEQ ID NO: 20 - protein, 256 aa, Artificial Sequence
  Description of Artificial Sequence: Synthetic polypeptide
GGPCRSHIDVAKPICVGGGGSGGLSGRSDAGSPLGLAGSGGSDILLTQSPVILSVSPGERVSFSCRASQSIGTNIHWYQQRTNGSPRLLIKYASESISGIPSRFSGSGSGTDFTLSINSVESEDIADYYCQQNNNWPTTFGAGTKLELKRTVAAPSVFIFPPSDEQLKSGTASVVCLLNNFYPREAKVQWKVDNALQSGNSQESVTEQDSKDSTYSLSSTLTLSKADYEKHKVYACEVTHQGLSSPVTKSFNRGEC

SEQ ID NO: 21 - protein, 660 aa, Artificial Sequence
  Description of Artificial Sequence: Synthetic polypeptide
EVQLVESGGGLVQPGNSLRLSCAASGFTFSKFGMSWVRQAPGKGLEWVSSISGSGRDTLYADSVKGRFTISRDNAKTTLYLQMNSLRPEDTAVYYCTIGGSLSVSSQGTLVTVSSGGGGSGGGSQGQSGQGYLWGCEWNCAGITTGSSGGSGGLSGRSDAGSPLGLAGSGGGSQTVVTQEPSLTVSPGGTVTLTCRSSTGAVTTSNYANWVQQKPGQAPRGLIGGTNKRAPGTPARFSGSLLGGKAALTLSGVQPEDEAEYYCALWYSNLWVFGGGTKLTVLGGGGSGGGGSGGGGSEVQLVESGGGLVQPGGSLKLSCAASGFTFNTYAMNWVRQAPGKGLEWVARIRSKYNNYATYYADSVKDRFTISRDDSKNTAYLQMNNLKTEDTAVYYCVRHGNFGNSYVSWFAYWGQGTLVTVSSGGGGSQVQLKQSGPGLVQPSQSLSITCTVSGFSLTNYGVHWVRQSPGKGLEWLGVIWSGGNTDYNTPFTSRLSINKDNSKSQVFFKMNSLQSNDTAIYYCARALTYYDYEFAYWGQGTLVTVSAASTKGPSVFPLAPSSKSTSGGTAALGCLVKDYFPEPVTVSWNSGALTSGVHTFPAVLQSSGLYSLSSVVTVPSSSLGTQTYICNVNHKPSNTKVDKKVEPKSCAAAHHHHHHHH

SEQ ID NO: 22 - protein, 214 aa, Artificial Sequence
  Description of Artificial Sequence: Synthetic polypeptide
QILLTQSPVILSVSPGERVSFSCRASQSIGTNIHWYQQRTNGSPRLLIKYASESISGIPSRFSGSGSGTDFTLSINSVESEDIADYYCQQNNNWPTTFGAGTKLELKRTVAAPSVFIFPPSDEQLKSGTASVVCLLNNFYPREAKVQWKVDNALQSGNSQESVTEQDSKDSTYSLSSTLTLSKADYEKHKVYACEVTHQGLSSPVTKSFNRGEC

SEQ ID NO: 23 - protein, 503 aa, Artificial Sequence
  Description of Artificial Sequence: Synthetic polypeptide
QTVVTQEPSLTVSPGGTVTLTCRSSTGAVTTSNYANWVQQKPGQAPRGLIGGTNKRAPGTPARFSGSLLGGKAALTLSGVQPEDEAEYYCALWYSNLWVFGGGTKLTVLGGGGSGGGGSGGGGSEVQLVESGGGLVQPGGSLKLSCAASGFTFNTYAMNWVRQAPGKGLEWVARIRSKYNNYATYYADSVKDRFTISRDDSKNTAYLQMNNLKTEDTAVYYCVRHGNFGNSYVSWFAYWGQGTLVTVSSGGGGSQVQLKQSGPGLVQPSQSLSITCTVSGFSLTNYGVHWVRQSPGKGLEWLGVIWSGGNTDYNTPFTSRLSINKDNSKSQVFFKMNSLQSQDTAIYYCARALTYYDYEFAYWGQGTLVTVSAASTKGPSVFPLAPSSKSTSGGTAALGCLVKDYFPEPVTVSWNSGALTSGVHTFPAVLQSSGLYSLSSVVTVPSSSLGTQTYICNVNHKPSNTKVDKKVEPKSCGGHHHHHHHHGGGLNDIFEAQKIEWHE

SEQ ID NO: 24 - protein, 214 aa, Artificial Sequence
  Description of Artificial Sequence: Synthetic polypeptide
DILLTQSPVILSVSPGERVSFSCRASQSIGTNIHWYQQRTNGSPRLLIKYASESISGIPSRFSGSGSGTDFTLSINSVESEDIADYYCQQNNNWPTTFGAGTKLELKRTVAAPSVFIFPPSDEQLKSGTASVVCLLNNFYPREAKVQWKVDNALQSGNSQESVTEQDSKDSTYSLSSTLTLSKADYEKHKVYACEVTHQGLSSPVTKSFNRGEC

SEQ ID NO: 25 - protein, 503 aa, Artificial Sequence
  Description of Artificial Sequence: Synthetic polypeptide
QTVVTQEPSLTVSPGGTVTLTCRSSTGAVTTSNYANWVQQKPGQAPRGLIGGTNKRAPGTPARFSGSLLGGKAALTLSGVQPEDEAEYYCALWYSNLWVFGGGTKLTVLGGGGSGGGGSGGGGSEVQLVESGGGLVQPGGSLKLSCAASGFTFNTYAMNWVRQAPGKGLEWVARIRSKYNNYATYYADSVKDRFTISRDDSKNTAYLQMNNLKTEDTAVYYCVRHGNFGNSYVSWFAYWGQGTLVTVSSGGGGSQVQLKQSGPGLVQPSQSLSITCTVSGFSLTNYGVHWVRQSPGKGLEWLGVIWSGGNTDYNTPFTSRLSINKDNSKSQVFFKMNSLQSNDTAIYYCARALTYYDYEFAYWGQGTLVTVSAASTKGPSVFPLAPSSKSTSGGTAALGCLVKDYFPEPVTVSWNSGALTSGVHTFPAVLQSSGLYSLSSVVTVPSSSLGTQTYICNVNHKPSNTKVDKKVEPKSCGGHHHHHHHHGGGLNDIFEAQKIEWHE

SEQ ID NO: 26 - protein, 17 aa, Artificial Sequence
  Description of Artificial Sequence: Synthetic peptide
AGLLAPPGGLSGRSDAG

SEQ ID NO: 27 - protein, 5 aa, Unknown
  Description of Unknown: Type I cytokine receptor sequence
  MOD_RES (3)..(3): Any amino acid
WSXWS